European Patent Application EP 4 331 616 A1, published March 6, 2024. Title: ANTIBODY DRUG CONJUGATE, PREPARATION METHOD THEREFOR AND APPLICATION THEREOF. Applicant: Tsinghua University Beijing Synthetic Vaccine Biosciences Co., Ltd. The sequence listing filed with the application follows.

SEQUENCE LISTING (9 sequences)

SEQ ID NO: 1 - DNA, 711 bp, Artificial Sequence
  Encoding Nucleotide of Light Chain of Avelumab
atggagacagacacactcctgctatgggtactgctgctctgggttccaggtagtaccggtcaatccgcactgactcaaccagccagcgttagcggctcccctggtcaatctatcaccatcagctgtaccgggaccagctcagacgttggcggttacaactacgtcagctggtaccagcagcacccgggtaaagctccaaagctgatgatttatgatgtgtctaatcgaccttctggtgtatctaaccgattttcaggctctaaaagtggaaatactgcttccctcacgatctcagggctgcaagccgaagacgaagccgattattattgttctagctatacatccagcagcacccgcgtgtttggaacgggaaccaaggtcacggttctgggacagcccaaagccaatcctaccgtcactctgttcccacccagtagtgaggagctgcaggcaaataaggctaccctggtctgtcttatatccgatttctatcccggggcagtcacagtcgcttggaaggcagatggctctccagtgaaggccggcgtcgaaacaactaaaccttccaagcagtctaataacaagtacgctgcttcttcttacctttcacttactcctgaacaatggaagagccacaggagttactcttgtcaggtaacccacgaggggtccactgtggagaaaaccgtcgctcccacagagtgttcttga

SEQ ID NO: 2 - DNA, 1413 bp, Artificial Sequence
  Encoding Nucleotide of Heavy Chain of Avelumab
atgtacaggatgcaactcctgtcttgcattgcactaagtcttgcacttgtcacgaattcggaagtacagctgcttgagagtggaggaggtttggtacagcccggcggatccctccgcctgtcctgtgcggctagtggctttacattctcatcctatatcatgatgtgggtaagacaggccccaggaaagggcctggagtgggttagttctatctacccctcaggcgggattaccttctacgcagatactgtgaagggcaggtttaccatatcccgagacaacagtaagaataccctttaccttcaaatgaactcccttcgggccgaggacactgcggtgtactattgcgctcgcattaagcttggcaccgtgacaaccgtgaactattggggtcaaggcacgctggtgactgtctcttccgcctccaccaagggcccatcggtcttccccctggcaccctcctccaagagcacctctgggggcacagcggccctgggctgcctggtcaaggactacttccccgaaccggtgacggtgtcgtggaactcaggcgccctgaccagcggcgtgcacaccttcccggctgtcctacagtcctcaggactctactccctcagcagcgtggtgactgtgccctctagcagcttgggcacccagacctacatctgcaacgtgaatcacaagcccagcaacaccaaggtggacaagaaagttgaacccaaatcttgcgacaaaactcacacatgcccaccgtgcccagcacctgaactcctggggggaccgtcagtcttcctcttccccccaaaacccaaggacaccctcatgatctcccggacccctgaggtcacatgcgtggtggtggacgtgagccacgaagaccctgaggtcaagttcaactggtacgtggacggcgtggaggtgcataatgccaagacaaagccgcgggaggagcagtacaacagcacgtaccgtgtggtcagcgtcctcaccgtcctgcaccaggactggctgaatggcaaggagtacaagtgcaaggtctccaacaaagccctcccagcccccatcgagaaaaccatctccaaagccaaagggcagccccgagaaccacaggtgtacaccctgcccccatcccgggatgagctgaccaagaaccaggtcagcctgacctgcctggtcaaaggcttctatcccagcgacatcgccgtggagtgggagagcaatgggcagccggagaacaactacaagaccacgcctcccgtgctggactccgacggctccttcttcctctacagcaagctcaccgtggacaagagcaggtggcagcaggggaacgtcttctcatgctccgtgatgcatgaggctctgcacaaccactacacgcagaagagcctctccctgtctccgggtaaatga

SEQ ID NO: 3 - protein, 236 aa, Artificial Sequence
  Light Chain of Avelumab
METDTLLLWVLLLWVPGSTGQSALTQPASVSGSPGQSITISCTGTSSDVGGYNYVSWYQQHPGKAPKLMIYDVSNRPSGVSNRFSGSKSGNTASLTISGLQAEDEADYYCSSYTSSSTRVFGTGTKVTVLGQPKANPTVTLFPPSSEELQANKATLVCLISDFYPGAVTVAWKADGSPVKAGVETTKPSKQSNNKYAASSYLSLTPEQWKSHRSYSCQVTHEGSTVEKTVAPTECS

SEQ ID NO: 4 - protein, 470 aa, Artificial Sequence
  Heavy Chain of Avelumab
MYRMQLLSCIALSLALVTNSEVQLLESGGGLVQPGGSLRLSCAASGFTFSSYIMMWVRQAPGKGLEWVSSIYPSGGITFYADTVKGRFTISRDNSKNTLYLQMNSLRAEDTAVYYCARIKLGTVTTVNYWGQGTLVTVSSASTKGPSVFPLAPSSKSTSGGTAALGCLVKDYFPEPVTVSWNSGALTSGVHTFPAVLQSSGLYSLSSVVTVPSSSLGTQTYICNVNHKPSNTKVDKKVEPKSCDKTHTCPPCPAPELLGGPSVFLFPPKPKDTLMISRTPEVTCVVVDVSHEDPEVKFNWYVDGVEVHNAKTKPREEQYNSTYRVVSVLTVLHQDWLNGKEYKCKVSNKALPAPIEKTISKAKGQPREPQVYTLPPSRDELTKNQVSLTCLVKGFYPSDIAVEWESNGQPENNYKTTPPVLDSDGSFFLYSKLTVDKSRWQQGNVFSCSVMHEALHNHYTQKSLSLSPGK

SEQ ID NO: 5 - DNA, 4143 bp, Unknown
  plasmid 159-pFuse-alphaPDL1-LC
ggatctgcgatcgctccggtgcccgtcagtgggcagagcgcacatcgcccacagtccccgagaagttggggggaggggtcggcaattgaacgggtgcctagagaaggtggcgcggggtaaactgggaaagtgatgtcgtgtactggctccgcctttttcccgagggtgggggagaaccgtatataagtgcagtagtcgccgtgaacgttctttttcgcaacgggtttgccgccagaacacagctgaagcttcgaggggctcgcatctctccttcacgcgcccgccgccctacctgaggccgccatccacgccggttgagtcgcgttctgccgcctcccgcctgtggtgcctcctgaactgcgtccgccgtctaggtaagtttaaagctcaggtcgagaccgggcctttgtccggcgctcccttggagcctacctagactcagccggctctccacgctttgcctgaccctgcttgctcaactctacgtctttgtttcgttttctgttctgcgccgttacagatccaagctgtgaccggcgcctacctgagatcaccggcgaaggagggccaccatggagacagacacactcctgctatgggtactgctgctctgggttccaggtagtaccggtcaatccgcactgactcaaccagccagcgttagcggctcccctggtcaatctatcaccatcagctgtaccgggaccagctcagacgttggcggttacaactacgtcagctggtaccagcagcacccgggtaaagctccaaagctgatgatttatgatgtgtctaatcgaccttctggtgtatctaaccgattttcaggctctaaaagtggaaatactgcttccctcacgatctcagggctgcaagccgaagacgaagccgattattattgttctagctatacatccagcagcacccgcgtgtttggaacgggaaccaaggtcacggttctgggacagcccaaagccaatcctaccgtcactctgttcccacccagtagtgaggagctgcaggcaaataaggctaccctggtctgtcttatatccgatttctatcccggggcagtcacagtcgcttggaaggcagatggctctccagtgaaggccggcgtcgaaacaactaaaccttccaagcagtctaataacaagtacgctgcttcttcttacctttcacttactcctgaacaatggaagagccacaggagttactcttgtcaggtaacccacgaggggtccactgtggagaaaaccgtcgctcccacagagtgttcttgataagtgctagctggccagacatgataagatacattgatgagtttggacaaaccacaactagaatgcagtgaaaaaaatgctttatttgtgaaatttgtgatgctattgctttatttgtaaccattataagctgcaataaacaagttaacaacaacaattgcattcattttatgtttcaggttcagggggaggtgtgggaggttttttaaagcaagtaaaacctctacaaatgtggtatggaattaattctaaaatacagcatagcaaaactttaacctccaaatcaagcctctacttgaatccttttctgagggatgaataaggcataggcatcaggggctgttgccaatgtgcattagctgtttgcagcctcaccttctttcatggagtttaagatatagtgtattttcccaaggtttgaactagctcttcatttctttatgttttaaatgcactgacctcccacattccctttttagtaaaatattcagaaataatttaaatacatcattgcaatgaaaataaatgttttttattaggcagaatccagatgctcaaggcccttcataatatcccccagtttagtagttggacttagggaacaaaggaacctttaatagaaattggacagcaagaaagcgagcttctagcttatcctcagtcctgctcctctgccacaaagtgcacgcagttgccggccgggtcgcgcagggcgaactcccgcccccacggctgctcgccgatctcggtcatggccggcccggaggcgtcccggaagttcgtggacacgacctccgaccactcggcgtacagctcgtccaggccgcgcacccacacccaggccagggtgttgtccggcaccacctggtcctggaccgcgctgatgaacagggtcacgtcgtcccggaccacaccggcgaagtcgtcctccacgaagtcccgggagaacccgagccggtcggtccagaactcgaccgctccggcgacgtcgcgcgcggtgagcaccggaacggcactggtcaacttggccatgatggctcctcctgtcaggagaggaaagagaagaaggttagtacaattgctatagtgagttgtattatactatgcagatatactatgccaatgattaattgtcaaactagggctgcagggttcatagtgccacttttcctgcactgccccatctcctgcccaccctttcccaggcatagacagtcagtgacttaccaaactcacaggagggagaaggcagaagcttgagacagacccgcgggaccgccgaactgcgaggggacgtggctagggcggcttcttttatggtgcgccggccctcggaggcagggcgctcggggaggcctagcggccaatctgcggtggcaggaggcggggccgaaggccgtgcctgaccaatccggagcacataggagtctcagccccccgccccaaagcaaggggaagtcacgcgcctgtagcgccagcgtgttgtgaaatgggggcttgggggggttggggccctgactagtcaaaacaaactcccattgacgtcaatggggtggagacttggaaatccccgtgagtcaaaccgctatccacgcccattgatgtactgccaaaaccgcatcatcatggtaatagcgatgactaatacgtagatgtactgccaagtaggaaagtcccataaggtcatgtactgggcataatgccaggcgggccatttaccgtcattgacgtcaatagggggcgtacttggcatatgatacacttgatgtactgccaagtgggcagtttaccgtaaatactccacccattgacgtcaatggaaagtccctattggcgttactatgggaacatacgtcattattgacgtcaatgggcgggggtcgttgggcggtcagccaggcgggccatttaccgtaagttatgtaacgcctgcaggttaattaagaacatgtgagcaaaaggccagcaaaaggccaggaaccgtaaaaaggccgcgttgctggcgtttttccataggctccgcccccctgacgagcatcacaaaaatcgacgctcaagtcagaggtggcgaaacccgacaggactataaagataccaggcgtttccccctggaagctccctcgtgcgctctcctgttccgaccctgccgcttaccggatacctgtccgcctttctcccttcgggaagcgtggcgctttctcatagctcacgctgtaggtatctcagttcggtgtaggtcgttcgctccaagctgggctgtgtgcacgaaccccccgttcagcccgaccgctgcgccttatccggtaactatcgtcttgagtccaacccggtaagacacgacttatcgccactggcagcagccactggtaacaggattagcagagcgaggtatgtaggcggtgctacagagttcttgaagtggtggcctaactacggctacactagaagaacagtatttggtatctgcgctctgctgaagccagttaccttcggaaaaagagttggtagctcttgatccggcaaacaaaccaccgctggtagcggtggtttttttgtttgcaagcagcagattacgcgcagaaaaaaaggatctcaagaagatcctttgatcttttctacggggtctgacgctcagtggaacgaaaactcacgttaagggattttggtcatggctagttaattaacatttaaatcagcggccgcaataaaatatctttattttcattacatctgtgtgttggttttttgtgtgaatcgtaactaacatacgctctccatcaaaacaaaacgaaacaaaacaaactagcaaaataggctgtccccagtgcaagtgcaggtgccagaacatttctctatcgaa

SEQ ID NO: 6 - DNA, 4845 bp, Unknown
  plasmid 162-pFuse-alphaPDL1-hIgG-Fc2
ggatctgcgatcgctccggtgcccgtcagtgggcagagcgcacatcgcccacagtccccgagaagttggggggaggggtcggcaattgaacgggtgcctagagaaggtggcgcggggtaaactgggaaagtgatgtcgtgtactggctccgcctttttcccgagggtgggggagaaccgtatataagtgcagtagtcgccgtgaacgttctttttcgcaacgggtttgccgccagaacacagctgaagcttcgaggggctcgcatctctccttcacgcgcccgccgccctacctgaggccgccatccacgccggttgagtcgcgttctgccgcctcccgcctgtggtgcctcctgaactgcgtccgccgtctaggtaagtttaaagctcaggtcgagaccgggcctttgtccggcgctcccttggagcctacctagactcagccggctctccacgctttgcctgaccctgcttgctcaactctacgtctttgtttcgttttctgttctgcgccgttacagatccaagctgtgaccggcgcctacctgagatcaccggcgaaggagggccaccatgtacaggatgcaactcctgtcttgcattgcactaagtcttgcacttgtcacgaattcggaagtacagctgcttgagagtggaggaggtttggtacagcccggcggatccctccgcctgtcctgtgcggctagtggctttacattctcatcctatatcatgatgtgggtaagacaggccccaggaaagggcctggagtgggttagttctatctacccctcaggcgggattaccttctacgcagatactgtgaagggcaggtttaccatatcccgagacaacagtaagaataccctttaccttcaaatgaactcccttcgggccgaggacactgcggtgtactattgcgctcgcattaagcttggcaccgtgacaaccgtgaactattggggtcaaggcacgctggtgactgtctcttccgcctccaccaagggcccatcggtcttccccctggcaccctcctccaagagcacctctgggggcacagcggccctgggctgcctggtcaaggactacttccccgaaccggtgacggtgtcgtggaactcaggcgccctgaccagcggcgtgcacaccttcccggctgtcctacagtcctcaggactctactccctcagcagcgtggtgactgtgccctctagcagcttgggcacccagacctacatctgcaacgtgaatcacaagcccagcaacaccaaggtggacaagaaagttgaacccaaatcttgcgacaaaactcacacatgcccaccgtgcccagcacctgaactcctggggggaccgtcagtcttcctcttccccccaaaacccaaggacaccctcatgatctcccggacccctgaggtcacatgcgtggtggtggacgtgagccacgaagaccctgaggtcaagttcaactggtacgtggacggcgtggaggtgcataatgccaagacaaagccgcgggaggagcagtacaacagcacgtaccgtgtggtcagcgtcctcaccgtcctgcaccaggactggctgaatggcaaggagtacaagtgcaaggtctccaacaaagccctcccagcccccatcgagaaaaccatctccaaagccaaagggcagccccgagaaccacaggtgtacaccctgcccccatcccgggatgagctgaccaagaaccaggtcagcctgacctgcctggtcaaaggcttctatcccagcgacatcgccgtggagtgggagagcaatgggcagccggagaacaactacaagaccacgcctcccgtgctggactccgacggctccttcttcctctacagcaagctcaccgtggacaagagcaggtggcagcaggggaacgtcttctcatgctccgtgatgcatgaggctctgcacaaccactacacgcagaagagcctctccctgtctccgggtaaatgataagtgctagctggccagacatgataagatacattgatgagtttggacaaaccacaactagaatgcagtgaaaaaaatgctttatttgtgaaatttgtgatgctattgctttatttgtaaccattataagctgcaataaacaagttaacaacaacaattgcattcattttatgtttcaggttcagggggaggtgtgggaggttttttaaagcaagtaaaacctctacaaatgtggtatggaattaattctaaaatacagcatagcaaaactttaacctccaaatcaagcctctacttgaatccttttctgagggatgaataaggcataggcatcaggggctgttgccaatgtgcattagctgtttgcagcctcaccttctttcatggagtttaagatatagtgtattttcccaaggtttgaactagctcttcatttctttatgttttaaatgcactgacctcccacattccctttttagtaaaatattcagaaataatttaaatacatcattgcaatgaaaataaatgttttttattaggcagaatccagatgctcaaggcccttcataatatcccccagtttagtagttggacttagggaacaaaggaacctttaatagaaattggacagcaagaaagcgagcttctagcttatcctcagtcctgctcctctgccacaaagtgcacgcagttgccggccgggtcgcgcagggcgaactcccgcccccacggctgctcgccgatctcggtcatggccggcccggaggcgtcccggaagttcgtggacacgacctccgaccactcggcgtacagctcgtccaggccgcgcacccacacccaggccagggtgttgtccggcaccacctggtcctggaccgcgctgatgaacagggtcacgtcgtcccggaccacaccggcgaagtcgtcctccacgaagtcccgggagaacccgagccggtcggtccagaactcgaccgctccggcgacgtcgcgcgcggtgagcaccggaacggcactggtcaacttggccatgatggctcctcctgtcaggagaggaaagagaagaaggttagtacaattgctatagtgagttgtattatactatgcagatatactatgccaatgattaattgtcaaactagggctgcagggttcatagtgccacttttcctgcactgccccatctcctgcccaccctttcccaggcatagacagtcagtgacttaccaaactcacaggagggagaaggcagaagcttgagacagacccgcgggaccgccgaactgcgaggggacgtggctagggcggcttcttttatggtgcgccggccctcggaggcagggcgctcggggaggcctagcggccaatctgcggtggcaggaggcggggccgaaggccgtgcctgaccaatccggagcacataggagtctcagccccccgccccaaagcaaggggaagtcacgcgcctgtagcgccagcgtgttgtgaaatgggggcttgggggggttggggccctgactagtcaaaacaaactcccattgacgtcaatggggtggagacttggaaatccccgtgagtcaaaccgctatccacgcccattgatgtactgccaaaaccgcatcatcatggtaatagcgatgactaatacgtagatgtactgccaagtaggaaagtcccataaggtcatgtactgggcataatgccaggcgggccatttaccgtcattgacgtcaatagggggcgtacttggcatatgatacacttgatgtactgccaagtgggcagtttaccgtaaatactccacccattgacgtcaatggaaagtccctattggcgttactatgggaacatacgtcattattgacgtcaatgggcgggggtcgttgggcggtcagccaggcgggccatttaccgtaagttatgtaacgcctgcaggttaattaagaacatgtgagcaaaaggccagcaaaaggccaggaaccgtaaaaaggccgcgttgctggcgtttttccataggctccgcccccctgacgagcatcacaaaaatcgacgctcaagtcagaggtggcgaaacccgacaggactataaagataccaggcgtttccccctggaagctccctcgtgcgctctcctgttccgaccctgccgcttaccggatacctgtccgcctttctcccttcgggaagcgtggcgctttctcatagctcacgctgtaggtatctcagttcggtgtaggtcgttcgctccaagctgggctgtgtgcacgaaccccccgttcagcccgaccgctgcgccttatccggtaactatcgtcttgagtccaacccggtaagacacgacttatcgccactggcagcagccactggtaacaggattagcagagcgaggtatgtaggcggtgctacagagttcttgaagtggtggcctaactacggctacactagaagaacagtatttggtatctgcgctctgctgaagccagttaccttcggaaaaagagttggtagctcttgatccggcaaacaaaccaccgctggtagcggtggtttttttgtttgcaagcagcagattacgcgcagaaaaaaaggatctcaagaagatcctttgatcttttctacggggtctgacgctcagtggaacgaaaactcacgttaagggattttggtcatggctagttaattaacatttaaatcagcggccgcaataaaatatctttattttcattacatctgtgtgttggttttttgtgtgaatcgtaactaacatacgctctccatcaaaacaaaacgaaacaaaacaaactagcaaaataggctgtccccagtgcaagtgcaggtgccagaacatttctctatcgaa

SEQ ID NO: 7 - DNA, 4143 bp, Unknown
  alphaPD-L1 THIOMAB LC-V205C
ggatctgcgatcgctccggtgcccgtcagtgggcagagcgcacatcgcccacagtccccgagaagttggggggaggggtcggcaattgaacgggtgcctagagaaggtggcgcggggtaaactgggaaagtgatgtcgtgtactggctccgcctttttcccgagggtgggggagaaccgtatataagtgcagtagtcgccgtgaacgttctttttcgcaacgggtttgccgccagaacacagctgaagcttcgaggggctcgcatctctccttcacgcgcccgccgccctacctgaggccgccatccacgccggttgagtcgcgttctgccgcctcccgcctgtggtgcctcctgaactgcgtccgccgtctaggtaagtttaaagctcaggtcgagaccgggcctttgtccggcgctcccttggagcctacctagactcagccggctctccacgctttgcctgaccctgcttgctcaactctacgtctttgtttcgttttctgttctgcgccgttacagatccaagctgtgaccggcgcctacctgagatcaccggcgaaggagggccaccatggagacagacacactcctgctatgggtactgctgctctgggttccaggtagtaccggtcaatccgcactgactcaaccagccagcgttagcggctcccctggtcaatctatcaccatcagctgtaccgggaccagctcagacgttggcggttacaactacgtcagctggtaccagcagcacccgggtaaagctccaaagctgatgatttatgatgtgtctaatcgaccttctggtgtatctaaccgattttcaggctctaaaagtggaaatactgcttccctcacgatctcagggctgcaagccgaagacgaagccgattattattgttctagctatacatccagcagcacccgcgtgtttggaacgggaaccaaggtcacggttctgggacagcccaaagccaatcctaccgtcactctgttcccacccagtagtgaggagctgcaggcaaataaggctaccctggtctgtcttatatccgatttctatcccggggcagtcacagtcgcttggaaggcagatggctctccagtgaaggccggcgtcgaaacaactaaaccttccaagcagtctaataacaagtacgctgcttcttcttacctttcacttactcctgaacaatggaagagccacaggagttactcttgtcaggtaacccacgaggggtccacttgcgagaaaaccgtcgctcccacagagtgttcttgataagtgctagctggccagacatgataagatacattgatgagtttggacaaaccacaactagaatgcagtgaaaaaaatgctttatttgtgaaatttgtgatgctattgctttatttgtaaccattataagctgcaataaacaagttaacaacaacaattgcattcattttatgtttcaggttcagggggaggtgtgggaggttttttaaagcaagtaaaacctctacaaatgtggtatggaattaattctaaaatacagcatagcaaaactttaacctccaaatcaagcctctacttgaatccttttctgagggatgaataaggcataggcatcaggggctgttgccaatgtgcattagctgtttgcagcctcaccttctttcatggagtttaagatatagtgtattttcccaaggtttgaactagctcttcatttctttatgttttaaatgcactgacctcccacattccctttttagtaaaatattcagaaataatttaaatacatcattgcaatgaaaataaatgttttttattaggcagaatccagatgctcaaggcccttcataatatcccccagtttagtagttggacttagggaacaaaggaacctttaatagaaattggacagcaagaaagcgagcttctagcttatcctcagtcctgctcctctgccacaaagtgcacgcagttgccggccgggtcgcgcagggcgaactcccgcccccacggctgctcgccgatctcggtcatggccggcccggaggcgtcccggaagttcgtggacacgacctccgaccactcggcgtacagctcgtccaggccgcgcacccacacccaggccagggtgttgtccggcaccacctggtcctggaccgcgctgatgaacagggtcacgtcgtcccggaccacaccggcgaagtcgtcctccacgaagtcccgggagaacccgagccggtcggtccagaactcgaccgctccggcgacgtcgcgcgcggtgagcaccggaacggcactggtcaacttggccatgatggctcctcctgtcaggagaggaaagagaagaaggttagtacaattgctatagtgagttgtattatactatgcagatatactatgccaatgattaattgtcaaactagggctgcagggttcatagtgccacttttcctgcactgccccatctcctgcccaccctttcccaggcatagacagtcagtgacttaccaaactcacaggagggagaaggcagaagcttgagacagacccgcgggaccgccgaactgcgaggggacgtggctagggcggcttcttttatggtgcgccggccctcggaggcagggcgctcggggaggcctagcggccaatctgcggtggcaggaggcggggccgaaggccgtgcctgaccaatccggagcacataggagtctcagccccccgccccaaagcaaggggaagtcacgcgcctgtagcgccagcgtgttgtgaaatgggggcttgggggggttggggccctgactagtcaaaacaaactcccattgacgtcaatggggtggagacttggaaatccccgtgagtcaaaccgctatccacgcccattgatgtactgccaaaaccgcatcatcatggtaatagcgatgactaatacgtagatgtactgccaagtaggaaagtcccataaggtcatgtactgggcataatgccaggcgggccatttaccgtcattgacgtcaatagggggcgtacttggcatatgatacacttgatgtactgccaagtgggcagtttaccgtaaatactccacccattgacgtcaatggaaagtccctattggcgttactatgggaacatacgtcattattgacgtcaatgggcgggggtcgttgggcggtcagccaggcgggccatttaccgtaagttatgtaacgcctgcaggttaattaagaacatgtgagcaaaaggccagcaaaaggccaggaaccgtaaaaaggccgcgttgctggcgtttttccataggctccgcccccctgacgagcatcacaaaaatcgacgctcaagtcagaggtggcgaaacccgacaggactataaagataccaggcgtttccccctggaagctccctcgtgcgctctcctgttccgaccctgccgcttaccggatacctgtccgcctttctcccttcgggaagcgtggcgctttctcatagctcacgctgtaggtatctcagttcggtgtaggtcgttcgctccaagctgggctgtgtgcacgaaccccccgttcagcccgaccgctgcgccttatccggtaactatcgtcttgagtccaacccggtaagacacgacttatcgccactggcagcagccactggtaacaggattagcagagcgaggtatgtaggcggtgctacagagttcttgaagtggtggcctaactacggctacactagaagaacagtatttggtatctgcgctctgctgaagccagttaccttcggaaaaagagttggtagctcttgatccggcaaacaaaccaccgctggtagcggtggtttttttgtttgcaagcagcagattacgcgcagaaaaaaaggatctcaagaagatcctttgatcttttctacggggtctgacgctcagtggaacgaaaactcacgttaagggattttggtcatggctagttaattaacatttaaatcagcggccgcaataaaatatctttattttcattacatctgtgtgttggttttttgtgtgaatcgtaactaacatacgctctccatcaaaacaaaacgaaacaaaacaaactagcaaaataggctgtccccagtgcaagtgcaggtgccagaacatttctctatcgaa

SEQ ID NO: 8 - DNA, 711 bp, Artificial Sequence
  Encoding Nucleotide of Light Chain of anti-PD-L1 THIOMAB
atggagacagacacactcctgctatgggtactgctgctctgggttccaggtagtaccggtcaatccgcactgactcaaccagccagcgttagcggctcccctggtcaatctatcaccatcagctgtaccgggaccagctcagacgttggcggttacaactacgtcagctggtaccagcagcacccgggtaaagctccaaagctgatgatttatgatgtgtctaatcgaccttctggtgtatctaaccgattttcaggctctaaaagtggaaatactgcttccctcacgatctcagggctgcaagccgaagacgaagccgattattattgttctagctatacatccagcagcacccgcgtgtttggaacgggaaccaaggtcacggttctgggacagcccaaagccaatcctaccgtcactctgttcccacccagtagtgaggagctgcaggcaaataaggctaccctggtctgtcttatatccgatttctatcccggggcagtcacagtcgcttggaaggcagatggctctccagtgaaggccggcgtcgaaacaactaaaccttccaagcagtctaataacaagtacgctgcttcttcttacctttcacttactcctgaacaatggaagagccacaggagttactcttgtcaggtaacccacgaggggtccacttgcgagaaaaccgtcgctcccacagagtgttcttga

SEQ ID NO: 9 - protein, 236 aa, Artificial Sequence
  Light chain of anti-PD-L1 THIOMAB
METDTLLLWVLLLWVPGSTGQSALTQPASVSGSPGQSITISCTGTSSDVGGYNYVSWYQQHPGKAPKLMIYDVSNRPSGVSNRFSGSKSGNTASLTISGLQAEDEADYYCSSYTSSSTRVFGTGTKVTVLGQPKANPTVTLFPPSSEELQANKATLVCLISDFYPGAVTVAWKADGSPVKAGVETTKPSKQSNNKYAASSYLSLTPEQWKSHRSYSCQVTHEGSTCEKTVAPTECS